European Patent Specification EP 3 541 944 B1, published July 29, 2026. Title: GENE EXPRESSION CASSETTE AND EXPRESSION VECTOR INCLUDING THE SAME. Applicant: CELL BIOTECH CO., LTD. The sequence listing filed with the application follows.

SEQUENCE LISTING (11 sequences)

SEQ ID NO: 1 - DNA, 324 bp, Artificial Sequence
  Promoter ChoS
ggatccgtgatgtacgtaagaaagatttacgtcaaatcacaacggccgtaggtgacggtggcgtcgctggacaacaagcgtatgaatatattcaagctttaaatgattaaagtcaaaataagccacggtgaaaaccggggcttttctttttgccaaaattcaaaaagtgattggtctatacctaaaattaaaaaaacgctttctggtattccatgggtattgtataatgaaagtaactataagttacatcataggaggacttttgaatgaaaaaaaagattatctcagctattttaatgtctacagtgatactttctgctgcag

SEQ ID NO: 2 - DNA, 184 bp, Artificial Sequence
  Promoter Erm
ggatcctttttagtatttttaattaattgtaatcagcacagttcattatcaaccaaacaaaaaataagtggttataatgaatcgttaataagcaaaattcatataaccaaattaaagagggttataatgaaaaaaaagattatctcagctattttaatgtctacagtgatactttctgctgcag

SEQ ID NO: 3 - DNA, 324 bp, Artificial Sequence
  Promoter PK
ggatccctaaagatcgcgttttagcaagtaagatgggtgcttacgctgttgagctactccttgaaggtaagggtggtttagcagttggaatcttagaaaataaggttcaagctcataacatgcttgacttgtttgatgcaaaacatcaagcagatgattcactttaccaattaagtgaagatttatcattctagagttctattaatatttggataaaatgacttaagaagtcttttataatttaaaatcaagggagagattctgtaatgaaaaaaaagattatctcagctattttaatgtctacagtgatactttctgctgcag

SEQ ID NO: 4 - DNA, 324 bp, Artificial Sequence
  Promoter GK
ggatccataatctggtaaattagttgagatggtattatgaaaacactttatgatgtgcaacaacttttaaagcaattcggaatatttgtttacgttggaaaacgtaaatgggatattgaattgatgagtattgaattgaaaaatttgtacaaagcaggagtcgtcgataaaccgacttatgttaaagctcagttggttttacgacatgagcatcatattgaagaggttagagataaccaacaaaaataatggagggtttcgaagtaatgaaaaaaaagattatctcagctattttaatgtctacagtgatactttctgctgcag

SEQ ID NO: 5 - DNA, 324 bp, Artificial Sequence
  Promoter G6Pi
ggatccatgccggctaaagtggtggataaattgaatcatccccaagaactggaataagataaaattgtagtgctttcaggctttaccagccatcttttgaaaaaattaatttctttcaaaagtgcgtgtgacaggtgatcaactagattaaatggggagggtatcccagtaaatattaggttaaatcggataggcttaaccaaattaagtaattttattgtataatggtacagataaagaattttaaacaaaaggggtagttattaatgaaaaaaaagattatctcagctattttaatgtctacagtgatactttctgctgcag

SEQ ID NO: 6 - DNA, 324 bp, Artificial Sequence
  Promoter 6PFK
ggatccccagttattttagtttatgaggatactaatgaacataatgagttgtctgaaaaattttatttaaatgacagttctgaagtaaaagaacaattagcagaattgctaggaagtcaacatatttcgttaattaaaaaataaattttgaataaagcacttacattcgattaattaagaaaatggtacagacaactgttttcaaaagtgataaaatcaacaatgaagttttgaaaaaactcaatatttctgtttgaggtgaaaagatgaaaaaaaagattatctcagctattttaatgtctacagtgatactttctgctgcag

SEQ ID NO: 7 - DNA, 324 bp, Artificial Sequence
  Promoter L-LDH
ggatcctcattttcatgttatttttccaccctcaacacgcaaaaacggctgaaagagcaaaaacccctcagctgtccacgtttattttcatgtaatattaccatattattgaccccaagcgggtcttttaacctctaacttatcaatcactttactaactatacccgaacttcataaaatttttactcaactttcttttatgaaaatgctatacttagtattgtttgataaattcaaatattatatgaaaaaaggggattgatcttatgaaaaaaaagattatctcagctattttaatgtctacagtgatactttctgctgcag

SEQ ID NO: 8 - DNA, 324 bp, Artificial Sequence
  Promoter D-LDH
ggatcccagttcaattaatttattttgaatcgtttgataatcagcatgacgcaatgtctgcagaatatcagttcaagcaacgaacgcgaagtagtaagattaaatttcttaaaaagaatggtatttcattaacaaatttaaaataatagtggtacagttaaggcaattaacgactaatttaatagcttgaatactgtaatattttttgaatcatgatacagtatgtaaaacaaattatttagccaagtctgagaggagaatttttgatgaaaaaaaagattatctcagctattttaatgtctacagtgatactttctgctgcag

SEQ ID NO: 9 - DNA, 4757 bp, Artificial Sequence
  Plasmid pCBT24-2
aagttaatgtaagccttaaggtttcaactaaagcaattacggtcaaccataaccatagtattggattgtcattttattggctataaaatagtaaatcagtgaatttcattggatccgctaaagatcgcgttttagcaagtaagatgggtgcttacgctgttgagctactccttgaaggtaagggtggtttagcagttggaatcttagaaaataaggttcaagctcataacatgcttgacttgtttgatgcaaaacatcaagcagatgattcactttaccaattaagtgaagatttatcattctagagttctattaatatttggataaaatgacttaagaagtcttttataatttaaaatcaagggagagattctgtaatgaaaaaaaagattatctcagctattttaatgtctacagtgatactttctgctgcagccccgttgtcaggtgtttacgctgaagtaattattatggctaccgttgatccagaaaagactctattccttgatgaaccaatgaataaagtttttgattggtctaacagtgaggctccggtgcgagatgccttatgggattactatatggaaaagaatagccgtgacacgatcaaaacagaagaagaaatgaaacctgtattagatatgtcagatgacgaagttaaagcattagcggagaaagtcttgaaaaagtaacctgacaagaaccagtctgctattgatagactatttttgtccgtgaaatcctcgcgtatttccgtgaggagcatagtatatttagcgatcttcaaattttaagtatattgattcatatgtttatcctcctaagtttgaggacaaatcggattccacggcctcaatgactgagctccgcctatttttataggttaatgtcatgataataatggtttcttagcgattcacaaaaaataggcacacgaaaaacaagttaagggatgcagtttatgcatcccttaacttacttattaaataatttatagctattgaaaagagataagaattgttcaaagctaatattgtttaaatcgtcaattcctgcatgttttaaggaattgttaaattgattttttgtaaatattttcttgtattctttgttaacccatttcataacgaaataattatacttttgtttatctttgtgtgatattcttgatttttttctacttaatctgataagtgagctattcactttaggtttaggatgaaaatattctcttggaaccatacttaatatagaaatatcaacttctgccattaaaagtaatgccaatgagcgttttgtatttaataatcttttagcaaacccgtattccacgattaaataaatctcattagctatactatcaaaaacaattttgcgtattatatccgtacttatgttataaggtatattaccatatattttataggattggtttttaggaaatttaaactgcaatatatccttgtttaaaacttggaaattatcgtgatcaacaagtttattttctgtagttttgcataatttatggtctatttcaatggcagttacgaaattacacctctttactaattcaagggtaaaatggccttttcctgagccgatttcaaagatattatcatgttcatttaatcttatatttgtcattattttatctatattatgttttgaagtaataaagttttgactgtgttttatatttttctcgttcattataaccctctttaatttggttatatgaattttgcttattaacgattcattataaccacttattttttgtttggttgataatgaactgtgctgattacaattaattaaaaatactaaaaatgcccatattttttcctccttataaaattagtataattatagcacgaaaaggatctaggtgaagatcctttttgataatctcatgaccaaaatcccttaacgtgagttttcgttccactgagcgtcagaccccgtagaaaagatcaaaggatcttcttgagatcctttttttctgcgcgtaatctgctgcttgcaaacaaaaaaaccaccgctaccagcggtggtttgtttgccggatcaagagctaccaactctttttccgaaggtaactggcttcagcagagcgcagataccaaatactgttcttctagtgtagccgtagttaggccaccacttcaagaactctgtagcaccgcctacatacctcgctctgctaatcctgttaccagtggctgctgccagtggcgataagtcgtgtcttaccgggttggactcaagacgatagttaccggataaggcgcagcggtcgggctgaacggggggttcgtgcacacagcccagcttggagcgaacgacctacaccgaactgagatacctacagcgtgagctatgagaaagcgccacgcttcccgaagggagaaaggcggacaggtatccggtaagcggcagggtcggaacaggagagcgcacgagggagcttccagggggaaacgcctggtatctttatagtcctgtcgggtttcgccacctctgacttgagcgtcgatttttgtgatgctcgtcaggggggcggagcctatggaaaaacgccagcaacgcggcctttttacggttcctggccttttgctggccttttgctcacatgttctttcctgcgttatcccctgattctgtggataaccgtattaccgcctttgagtgagctgataccgctcgccgcagccgaacgaccgagcgcagcgagtcagtgagcgaggaaatcgatactgaattggcgaaagccaaagtttctataaaaccttgctttcctgcttaacggcgagtgaaaaagcggttaagctggctcagcttggacggggttcggggcgttagcgtccgtattaaatgtggcttaccataaccaacgaacagagtgaggtgcaaggagctgtgcgactggagtttaatgtgagccggtttttggctcactcctttgtgttttttgtttctagattttaatctcgtacagcggtgcctcttttatacctcttttataaacctcttttaaacctcttttagacccctcttgagccttactctcccaaggctcacagaaggttatcaagtaccttttgtctgtttatcaagtaccttttgtctgtttatcaagtaccttttgtctgtttatcaagtaccttttgtctgtttatcaagtacctttataagttctgtacttgataaaaaggtacttttattttaatatgtgtttgaggtgataatcatggctaatgagttagttaagtatgatcctgagttgaatactattcccttgagaaaatttaccccaattgagatgaatttatttttttcaattatttcccgcatgcgggatcaagggaataaaactgttcgtttctcttttgaccagttaaaagagcttagtaactataaaccaaccgcaaataaacgttttattgatgatattgaaaatacataccaaaagatcctcagccttaggtttggccgtagaagtaagagtggcttaaatcgtgaattttttgttatgtttactgaatttgaaattaaaggtgaagctgaagaaccttatgttgatattcagatttatcccaaagcattgcacttgctaaacgatttagaaagttgggttcgttatgccctaacagaatttagaaatttaaaaagcagttacgctaaaacaatgtttcgtctaattaagcaatttcgaactactggctattcttatttctctaaagaagatttttttgaattgcttgatatacctaaaagttattggaatagtccttcaaaggttgacaaaaaggttattaagccaattagagaagaattaaccccgctttttagagggctaacgattagaaaaaaatatggtaaaggcagaggaaaaccagttatcggttattcttttacttggaaacctgaaagcaaggacgcaaatgatttttctcaaggcaaatttcaagatgagcgtcaaaaactctttaacattcagcacaatgatgaattatcagataaagaaaagtggcgtgcaattgacaaagttaaatgcttgcctttaggaacaactgaaaaacaggtactggctgaaaaacaagctgaacatgatcaaaaaatcagagatcaagcaagacaagaatttctcgctgatctccgaaaggggttttaaaatcatgtctaaaactattagagaacttgctgatgaattgaatgtctccaaacagactattcaatatcactaccaaagactaccagcaaagaaccaacaaaagaatagtcagggcacaaaccttattagtcctacagcagaaagaattataagaagcaaggtagcaaagcctttgctagcaaaaaaacagcaaagaggtagcaaagaattgccaaagactagcaaagaaaataatgatctggttgctactctgagaagagaagtagaagatttaaaggctcaacgtgacaaacagcttgctaccaaagaccgacaaatagaccatctaacaaaattggtggatcagcagcaacaattacaattagcaacagtagcagataaccgtcgattaaaagatcatgtacaaaagctaagtgggcaactaactcaaaaaactaacgacaacttgtcgaccggaaatgatctttttaacatccaagataaagaaagcaaaatagctaaacagaagattgttaaatctggtagtaataaagatggcatacacacaaatagagctattaaacgttggtggaaattctggtaa

SEQ ID NO: 10 - protein, 234 aa, Artificial Sequence
  P8 protein
GAAGTAATTATTATGGCTACCGTTGATCCAGAAAAGACTCTATTCCTTGATGAACCAATGAATAAAGTTTTTGATTGGTCTAACAGTGAGGCTCCGGTGCGAGATGCCTTATGGGATTACTATATGGAAAAGAATAGCCGTGACACGATCAAAACAGAAGAAGAAATGAAACCTGTATTAGATATGTCAGATGACGAAGTTAAAGCATTAGCGGAGAAAGTCTTGAAAAAGTAA

SEQ ID NO: 11 - protein, 122 aa, Artificial Sequence
  p14 Protein
AKSQDQFNEKAGKKITVSDEAVDKAAKKIEQVGYVTEKDVPEMIDRDYTRALSKKVSAKLHQDKDDDYFYEEPFDYENGRIANIIWDMDKIKTREEAMKTLANELGLTVPKIVMRKVDEQVF